European Patent Specification EP 3 899 035 B1, published April 16, 2025. Title: DETECTION OF TARGET NUCLEIC ACID BY SOLID-PHASE MOLOGRAPHY. Applicant: F. Hoffmann-La Roche AG Roche Diagnostics GmbH Roche Molecular Systems, Inc. The sequence listing filed with the application follows.

SEQUENCE LISTING (4 sequences)

SEQ ID NO: 1 - DNA, 49 bp, Artificial Sequence
  HIV-1 LTR tag 3 probe
cacacattggcaccgccgtcttctctagcagtggcgcccgaacagggac

SEQ ID NO: 2 - DNA, 38 bp, Artificial Sequence
  Moligo tag 3 oligonucleotide
ttttttttttttagagaagacggcggtgccaatgtgtg

SEQ ID NO: 3 - DNA, 22 bp, Artificial Sequence
  AT-MOLO-3 oligonucleotide
cacacattggcaccgccgtctt

SEQ ID NO: 4 - DNA, 100 bp, Artificial Sequence
  HIV-LTR-moligo-100 oligonucleotide
ttgcatgagaatagtaacgtattgtgtaaagcaggatatagagtaattgcccagttgttccaaatcgatattgcagagaagacggcggtgccaatgtgtg